European Patent Application EP 4 420 675 A1, published August 28, 2024. Title: Epitope modification. Applicant: NANTONG YICHEN BIOPHARMA. CO. LTD. The sequence listing filed with the application follows.

SEQUENCE LISTING (32 sequences)

SEQ ID NO: 1 - DNA, 459 bp, synthetic construct
  source 1..459: mol_type = other DNA
gcgcctgtgcggagcctgaactgtacccttcgggattcccaacagaaaagcttagtgatgagtggaccgtatgaactgaaggctttgcatctgcagggacaggacatggaacaacaagttgttttctcaatgtcattcgtacagggtgaggagtccaatgataaaatcccagtagcattgggccttaaggagaagaatctgtacctgagctgtgtactgaaagacgataagccgacactccaactggaaagtgtggacccgaagaattatccgaaaaaaaaaatggaaaagcgctttgtttttaacaaaatcgaaatcaacaacaaattagaatttgagtcggcgcagtttccgaactggtatatcagcacgtctcaggcggaaaacatgccagtgttcttaggtggtaccaaaggaggtcaagatattacggactttacgatgcagttcgtgtcatcg

SEQ ID NO: 2 - protein, 153 aa, synthetic construct
APVRSLNCTLRDSQQKSLVMSGPYELKALHLQGQDMEQQVVFSMSFVQGEESNDKIPVALGLKEKNLYLSCVLKDDKPTLQLESVDPKNYPKKKMEKRFVFNKIEINNKLEFESAQFPNWYISTSQAENMPVFLGGTKGGQDITDFTMQFVSS

SEQ ID NO: 3 - DNA, 321 bp, synthetic construct
  source 1..321: mol_type = other DNA
gacattgtaatgacccagtctcaaaaattcatgtccacatcagtaggagacagggtcagcatcacctgcaaggccagtcagaatgttcgtactgctgtagcctggtatcaacagaaaccaggccagtctcctaaagcactgatttacttggcatccaaccgacacactggagtccctgatcgcttcacaggcagtggatctgggacagatttcactctcaccattaccaatgtgcaatctgaagacctggcagattatttctgtctgcaacattggaattatcctctcacattcggtgctgggaccaagctggagctgaaa

SEQ ID NO: 4 - protein, 107 aa, synthetic construct
DIVMTQSQKFMSTSVGDRVSITCKASQNVRTAVAWYQQKPGQSPKALIYLASNRHTGVPDRFTGSGSGTDFTLTITNVQSEDLADYFCLQHWNYPLTFGAGTKLELK

SEQ ID NO: 5 - DNA, 354 bp, synthetic construct
  source 1..354: mol_type = other DNA
gaggtgcagctgaaggagtctggagctgagctgatgaagcctggggcctcagtgaagatatcctgcaaggctactggctacacattcagtagctactggatagagtgggtaaagcagaggcctggacatggccttgagtggattggagagattttacctggaagtggtagtactaactacaatgagaagttcaagggcaaggccacattcactgcagatatatcctccaacacagcctacatgcaactcagcagcctgacatctgaggactctgccgtctattactgtgcaagtgggggatatagaccctctatggacttctggggtcaaggaacctcagtcaccgtctcctca

SEQ ID NO: 6 - protein, 118 aa, synthetic construct
EVQLKESGAELMKPGASVKISCKATGYTFSSYWIEWVKQRPGHGLEWIGEILPGSGSTNYNEKFKGKATFTADISSNTAYMQLSSLTSEDSAVYYCASGGYRPSMDFWGQGTSVTVSS

SEQ ID NO: 7 - DNA, 321 bp, synthetic construct
  source 1..321: mol_type = other DNA
gatattgtaatgacccagtctcaaaaattcatgtccacatcagtaggagacagggtcagcatcacctgccaggccagtcagaatgttcgtactgctgtagcctggtaccaacagaaaccagggcagtctccaaaagcactgatttactcggcatcctcccggtacagtggagtccctgatcgcttcacaggcagtggatctgggacagatttcactctcaccatcagcaatgtgcagtctgaagacttggcagagtatttctgtcagcaatataacagctatcctctcacgttcggtgctgggaccaagctggagctgaaa

SEQ ID NO: 8 - protein, 107 aa, synthetic construct
DIVMTQSQKFMSTSVGDRVSITCQASQNVRTAVAWYQQKPGQSPKALIYSASSRYSGVPDRFTGSGSGTDFTLTISNVQSEDLAEYFCQQYNSYPLTFGAGTKLELK

SEQ ID NO: 9 - DNA, 351 bp, synthetic construct
  source 1..351: mol_type = other DNA
gaggtccagctccagcaatctggggcagagcttgtgaaggcgggggcctcagtcaagttgtcctgcacagcttctggcttcaacattacagacacctatattcactgggtgaagcagaggcctgaacagggcctggagtggattggaaggattgatcctgcgaatggtaatactaaatatgacccgaagttccagggcaaggccactataacatcagacacatcctccaacacagcctacttgcagctcagcagcctgacatctgaggacactgccgtctattactgtcctcttcattactacggctggtttatttactggggccaagggactctggtcactgtctctgca

SEQ ID NO: 10 - protein, 117 aa, synthetic construct
EVQLQQSGAELVKAGASVKLSCTASGFNITDTYIHWVKQRPEQGLEWIGRIDPANGNTKYDPKFQGKATITSDTSSNTAYLQLSSLTSEDTAVYYCPLHYYGWFIYWGQGTLVTVSA

SEQ ID NO: 11 - DNA, 321 bp, synthetic construct
  source 1..321: mol_type = other DNA
gatattgtaatgacccaatctcaaaaattcatgtccacatcagtaggagacagggtcagcatcacctgcaaggccagtcagaatgttcgtactgctgtagcctggtatcaacagaaaccagggcagtctcctaaagcactgatttacttggcatccaaccgacacactggagtccctgatcgcttcacaggcagtggatctgggacagatttcactctcaccattaccaatgtgcaatctgaagacctggcagattatttctgtctgcaacattggaattatcctctcacgttcggtgctgggaccaagctggagctgaaa

SEQ ID NO: 12 - protein, 107 aa, synthetic construct; identical to SEQ ID NO: 4

SEQ ID NO: 13 - DNA, 369 bp, synthetic construct
  source 1..369: mol_type = other DNA
gaggtgcagctggtggagtcaggacctggcctggtggcaccctcacagagcctgtccatcacatgcactgtctctgggttctcattatccagatatagtgtacactgggttcgccagcctccaggaaggggtctggagtggctgggagtgatatggggtggtggaggcacagactataattcagctctcaaatccagactgagcatcagcaaggacaactccaagagccaagttttcttaaaaatgaacagtctgcaaactgatgacacagccatgtactactgtgccagaaatacgaattactacggtagtacttacgaccatgctatggactactggggtcaaggaacctcagtcaccgtctcctca

SEQ ID NO: 14 - protein, 123 aa, synthetic construct
EVQLVESGPGLVAPSQSLSITCTVSGFSLSRYSVHWVRQPPGRGLEWLGVIWGGGGTDYNSALKSRLSISKDNSKSQVFLKMNSLQTDDTAMYYCARNTNYYGSTYDHAMDYWGQGTSVTVSS

SEQ ID NO: 15 - DNA, 321 bp, synthetic construct
  source 1..321: mol_type = other DNA
ggtattgtaatgacccagtctcacaaattcatgtccacatcagtaggagacagggtcagcatcacctgcaaggccagtcaggatgtgggtactgctgtagcctggtatcaacagaaaccagggcaatctcctaaactactgatttactgggcatccacccggcacactggagtccctgatcgcttcacaggcagtggatctgggacagatttcactctcaccattagcaatgtgcagtctgaagacttggcagattatttctgtcagcaatatagcagctatccgctcacgttcggtgctgggaccatgctggagctgaaa

SEQ ID NO: 16 - protein, 107 aa, synthetic construct
GIVMTQSHKFMSTSVGDRVSITCKASQDVGTAVAWYQQKPGQSPKLLIYWASTRHTGVPDRFTGSGSGTDFTLTISNVQSEDLADYFCQQYSSYPLTFGAGTMLELK

SEQ ID NO: 17 - DNA, 351 bp, synthetic construct
  source 1..351: mol_type = other DNA
gaggtgcagcttcagcagtctggggcagagcttgtgaagccaggggcctcagtcaagttgtcctgcacagcttctggcttcaacattaaagacacctatatgcactgggtgaagcagaggcctgaacagggcctggagtggattggaaggattgatcctgcgaatggtaatactaaatatgacccgaagttccagggcaaggccactataacagcagacacgtcctccaacacagcctacctgcagctcagcagcctgacatctgaggacactgccgtctattactgtgccatccattactacggtagtctccctgtctggggcgcagggaccacggtcaccgtctcctca

SEQ ID NO: 18 - protein, 117 aa, synthetic construct
EVQLQQSGAELVKPGASVKLSCTASGFNIKDTYMHWVKQRPEQGLEWIGRIDPANGNTKYDPKFQGKATITADTSSNTAYLQLSSLTSEDTAVYYCAIHYYGSLPVWGAGTTVTVSS

SEQ ID NO: 19 - DNA, 321 bp, synthetic construct
  source 1..321: mol_type = other DNA
gacattaagataacccagtctccagcctccctatctgcatctgtgggagaaactgtcaccatcacatgtcgagcaagtgagaatatttacagttatttagcatggtatcagcagaaacagggaaaatctcctcagctcctggtctataatgcaaaaaccttagcagaaggtgtgccatcaaggttcagtggcagtggatcaggcacacagttttctctgaagatcaacagcctgcagcctgaagattttgggagttattactgtcaacatcattatggtactccgctcacgttcggtgctgggaccaagctggaaatcaaa

SEQ ID NO: 20 - protein, 107 aa, synthetic construct
DIKITQSPASLSASVGETVTITCRASENIYSYLAWYQQKQGKSPQLLVYNAKTLAEGVPSRFSGSGSGTQFSLKINSLQPEDFGSYYCQHHYGTPLTFGAGTKLEIK

SEQ ID NO: 21 - DNA, 363 bp, synthetic construct
  source 1..363: mol_type = other DNA
gaggtgcagctggtggagtctgggggaggcttagtgcagcctggagggtcccggaaactctcctgtgcagcctctggattcactttcagtagctttggaatgcactgggttcgtcaggctccagagaaggggctggagtgggtcgcatacattagtagtggcagtagtaccatctactatgcagacacagtgaagggccgattcaccatctccagagacaatcccaagaacaccctgttcctgcaaatgaccagtctaaggtctgaggacacggccatgtattactgtgcaagagacgattacgacgtgagggcctatgctatggactactggggtcaaggaacctcagtcaccgtctcctca

SEQ ID NO: 22 - protein, 121 aa, synthetic construct
EVQLVESGGGLVQPGGSRKLSCAASGFTFSSFGMHWVRQAPEKGLEWVAYISSGSSTIYYADTVKGRFTISRDNPKNTLFLQMTSLRSEDTAMYYCARDDYDVRAYAMDYWGQGTSVTVSS

SEQ ID NO: 23 - DNA, 321 bp, synthetic construct
  source 1..321: mol_type = other DNA
gacattgtgatgacacaaccttcatcctccttttctgtatctctaggagacagagtcaccattacttgcaaggcaagtgaggacatatataatcggttagcctggtatcagcagaaaccaggaaatgctcctaggctcttaatatctggtgcaaccactttggaaactggggttccttcaagattcagtggcagtggatctggaaaggattacactctcaccattaccagtcttcagactgaagatgttgctacttattactgtcaacagtattggagtactccgctcacgttcggtgctgggaccaagctggagctgaaa

SEQ ID NO: 24 - protein, 107 aa, synthetic construct
DIVMTQPSSSFSVSLGDRVTITCKASEDIYNRLAWYQQKPGNAPRLLISGATTLETGVPSRFSGSGSGKDYTLTITSLQTEDVATYYCQQYWSTPLTFGAGTKLELK

SEQ ID NO: 25 - DNA, 363 bp, synthetic construct
  source 1..363: mol_type = other DNA
gaggtgcagctggtggagtctgggggaggcttagtgcagcctggagggtcccggaaactctcctgtgcagcctctggattcactttcagtagctttggaatgcactgggttcgtcaggctccagagaaggggctggagtgggtcgcatacattagtagtggcagttataccatctactatgcagacacagtgaagggccgattcaccatctccagagacaatcccaagaacaccctgttcctgcaaatgaccagtctaaggtctgaggacacggccatgtattactgtacaagagacgattacgacgtgagggcctatgctatggactactggggtcaaggaacctcagtcaccgtctcctca

SEQ ID NO: 26 - protein, 121 aa, synthetic construct
EVQLVESGGGLVQPGGSRKLSCAASGFTFSSFGMHWVRQAPEKGLEWVAYISSGSYTIYYADTVKGRFTISRDNPKNTLFLQMTSLRSEDTAMYYCTRDDYDVRAYAMDYWGQGTSVTVSS

SEQ ID NO: 27 - DNA, 321 bp, synthetic construct
  source 1..321: mol_type = other DNA
gatattgtgatgactcaggctcacaaattcatgtccacatcagtaggagacagggtcagcatcacctgccaggccagtcaggatgtgggtactgctgtagcctggtatcaacagaaaccagggcaatctcctaaactactgatttactgggcatccacccggcacactggagtccctgatcgcttcacaggcagtggatctgggacagatttcactctcaccattagcaatgtgcagtctgaagacttggcagattatttctgtcagcaatatagcagctatccgtacacgttcggaggggggaccaagctggaaataaaa

SEQ ID NO: 28 - protein, 107 aa, synthetic construct
DIVMTQAHKFMSTSVGDRVSITCQASQDVGTAVAWYQQKPGQSPKLLIYWASTRHTGVPDRFTGSGSGTDFTLTISNVQSEDLADYFCQQYSSYPYTFGGGTKLEIK

SEQ ID NO: 29 - DNA, 351 bp, synthetic construct
  source 1..351: mol_type = other DNA
gaggttcagcttcagcagtctggggcagagcttgtgaagccaggggcctcagtcaagttgtcctgcacagcttctgacttcaacattaaagacacctatatacactgggtgaagcagaggcctgaacagggcctcgagtggattggaaggattgatcctgcggatggtaatactaaatatgacccgaagttccagggcaaggccactataacagcagacacatcctccaacacagcctacctgcagctcagcagcctgacatctgaggacactgccgtctattactgtgccattcattactacggctcgtttccttactggggccaagggactctggtcactgtctctgca

SEQ ID NO: 30 - protein, 117 aa, synthetic construct
EVQLQQSGAELVKPGASVKLSCTASDFNIKDTYIHWVKQRPEQGLEWIGRIDPADGNTKYDPKFQGKATITADTSSNTAYLQLSSLTSEDTAVYYCAIHYYGSFPYWGQGTLVTVSA

SEQ ID NO: 31 - DNA, 642 bp, synthetic construct
  source 1..642: mol_type = other DNA
gacaaaactcacacatgcgtcttcatcttccctccaaagatcaaggatgtactcatgatctccctgagccccatagtcacatgtgtggtggtggatgtgagcgaggatgacccagatgtccagatcagctggtttgtgaacaacgtggaagtacacacagctcagacacaaacccatagagaggattacaacagtactctccgggtggtcagtgccctccccatccagcaccaggactggatgagtggcaaggagttcaaatgcaaggtcaacaacaaagacctcccagcgcccatcgagagaaccatctcaaaacccaaagggtcagtaagagctccacaggtatatgtcttgcctccaccagaagaagagatgactaagaaacaggtcactctgacctgcatggtcacagacttcatgcctgaagacatttacgtggagtggaccaacaacgggaaaacagagctaaactacaagaacactgaaccagtcctggactctgatggttcttacttcatgtacagcaagctgagagtggaaaagaagaactgggtggaaagaaatagctactcctgttcagtggtccacgagggtctgcacaatcaccacacgactaagagcttctcccggactccgggtaaa

SEQ ID NO: 32 - protein, 214 aa, synthetic construct
DKTHTCVFIFPPKIKDVLMISLSPIVTCVVVDVSEDDPDVQISWFVNNVEVHTAQTQTHREDYNSTLRVVSALPIQHQDWMSGKEFKCKVNNKDLPAPIERTISKPKGSVRAPQVYVLPPPEEEMTKKQVTLTCMVTDFMPEDIYVEWTNNGKTELNYKNTEPVLDSDGSYFMYSKLRVEKKNWVERNSYSCSVVHEGLHNHHTTKSFSRTPGK